European Patent Specification EP 3 626 262 B1, published October 23, 2024. Title: VEGFR-2 targeting DNA Vaccine for Combination Therapy. Applicant: VAXIMM AG. The sequence listing filed with the application follows.

SEQUENCE LISTING (15 sequences)

SEQ ID NO: 1 - protein, 1356 aa, human
MQSKVLLAVALWLCVETRAASVGLPSVSLDLPRLSIQKDILTIKANTTLQITCRGQRDLDWLWPNNQSGSEQRVEVTECSDGLFCKTLTIPKVIGNDTGAYKCFYRETDLASVIYVYVQDYRSPFIASVSDQHGVVYITENKNKTVVIPCLGSISNLNVSLCARYPEKRFVPDGNRISWDSKKGFTIPSYMISYAGMVFCEAKINDESYQSIMYIVVVVGYRIYDVVLSPSHGIELSVGEKLVLNCTARTELNVGIDFNWEYPSSKHQHKKLVNRDLKTQSGSEMKKFLSTLTIDGVTRSDQGLYTCAASSGLMTKKNSTFVRVHEKPFVAFGSGMESLVEATVGERVRIPAKYLGYPPPEIKWYKNGIPLESNHTIKAGHVLTIMEVSERDTGNYTVILTNPISKEKQSHVVSLVVYVPPQIGEKSLISPVDSYQYGTTQTLTCTVYAIPPPHHIHWYWQLEEECANEPSQAVSVTNPYPCEEWRSVEDFQGGNKIEVNKNQFALIEGKNKTVSTLVIQAANVSALYKCEAVNKVGRGERVISFHVTRGPEITLQPDMQPTEQESVSLWCTADRSTFENLTWYKLGPQPLPIHVGELPTPVCKNLDTLWKLNATMFSNSTNDILIMELKNASLQDQGDYVCLAQDRKTKKRHCVVRQLTVLERVAPTITGNLENQTTSIGESIEVSCTASGNPPPQIMWFKDNETLVEDSGIVLKDGNRNLTIRRVRKEDEGLYTCQACSVLGCAKVEAFFIIEGAQEKTNLEIIILVGTAVIAMFFWLLLVIILRTVKRANGGELKTGYLSIVMDPDELPLDEHCERLPYDASKWEFPRDRLKLGKPLGRGAFGQVIEADAFGIDKTATCRTVAVKMLKEGATHSEHRALMSELKILIHIGHHLNVVNLLGACTKPGGPLMVIVEFCKFGNLSTYLRSKRNEFVPYKTKGARFRQGKDYVGAIPVDLKRRLDSITSSQSSASSGFVEEKSLSDVEEEEAPEDLYKDFLTLEHLICYSFQVAKGMEFLASRKCIHRDLAARNILLSEKNVVKICDFGLARDIYKDPDYVRKGDARLPLKWMAPETIFDRVYTIQSDVWSFGVLLWEIFSLGASPYPGVKIDEEFCRRLKEGTRMRAPDYTTPEMYQTMLDCWHGEPSQRPTFSELVEHLGNLLQANAQQDGKDYIVLPISETLSMEEDSGLSLPTSPVSCMEEEEVCDPKFHYDNTAGISQYLQNSKRKSRPVSVKTFEDIPLEEPEVKVIPDDNQTDSGMVLASEELKTLEDRTKLSPSFGGMVPSKSRESVASEGSNQTSGYQSGYHSDDTDTTVYSSEEAELLKLIEIGVQTGSTAQILQPDSGTTLSSPPV

SEQ ID NO: 2 - DNA, 3500 bp, artificial
  expression plasmid
tgggcttttgctggccttttgctcacatgttcttgactcttcgcgatgtacgggccagatatacgcgttgacattgattattgactagttattaatagtaatcaattacggggtcattagttcatagcccatatatggagttccgcgttacataacttacggtaaatggcccgcctggctgaccgcccaacgacccccgcccattgacgtcaataatgacgtatgttcccatagtaacgccaatagggactttccattgacgtcaatgggtggactatttacggtaaactgcccacttggcagtacatcaagtgtatcatatgccaagtacgccccctattgacgtcaatgacggtaaatggcccgcctggcattatgcccagtacatgaccttatgggactttcctacttggcagtacatctacgtattagtcatcgctattaccatggtgatgcggttttggcagtacatcaatgggcgtggatagcggtttgactcacggggatttccaagtctccaccccattgacgtcaatgggagtttgttttggcaccaaaatcaacgggactttccaaaatgtcgtaacaactccgccccattgacgcaaatgggcggtaggcgtgtacggtgggaggtctatataagcagagctctctggctaactagagaacccactgcttactggcttatcgaaattaatacgactcactatagggagacccaagctggctagcctcgagtctagagggcccgtttaaacccgctgatcagcctcgactgtgccttctagttgccagccatctgttgtttgcccctcccccgtgccttccttgaccctggaaggtgccactcccactgtcctttcctaataaaatgaggaaattgcatcgcattgtctgagtaggtgtcattctattctggggggtggggtggggcaggacagcaagggggaggattgggaagacaatagcaggcatgctggggatgcggtgggctctatggcttctactgggcggttttatggacagcaagcgaaccggaattgccagctggggcgccctctggtaaggttgggaagccctgcaaagtaaactggatggctttctcgccgccaaggatctgatggcgcaggggatcaagctctgatcaagagacaggatgaggatcgtttcgcatgattgaacaagatggattgcacgcaggttctccggccgcttgggtggagaggctattcggctatgactgggcacaacagacaatcggctgctctgatgccgccgtgttccggctgtcagcgcaggggcgcccggttctttttgtcaagaccgacctgtccggtgccctgaatgaactgcaagacgaggcagcgcggctatcgtggctggccacgacgggcgttccttgcgcagctgtgctcgacgttgtcactgaagcgggaagggactggctgctattgggcgaagtgccggggcaggatctcctgtcatctcaccttgctcctgccgagaaagtatccatcatggctgatgcaatgcggcggctgcatacgcttgatccggctacctgcccattcgaccaccaagcgaaacatcgcatcgagcgagcacgtactcggatggaagccggtcttgtcgatcaggatgatctggacgaagagcatcaggggctcgcgccagccgaactgttcgccaggctcaaggcgagcatgcccgacggcgaggatctcgtcgtgacccatggcgatgcctgcttgccgaatatcatggtggaaaatggccgcttttctggattcatcgactgtggccggctgggtgtggcggaccgctatcaggacatagcgttggctacccgtgatattgctgaagagcttggcggcgaatgggctgaccgcttcctcgtgctttacggtatcgccgctcccgattcgcagcgcatcgccttctatcgccttcttgacgagttcttctgaattattaacgcttacaatttcctgatgcggtattttctccttacgcatctgtgcggtatttcacaccgcatacaggtggcacttttcggggaaatgtgcgcggaacccctatttgtttatttttctaaatacattcaaatatgtatccgctcatgagacaataaccctgataaatgcttcaataatagcacgtgctaaaacttcatttttaatttaaaaggatctaggtgaagatcctttttgataatctcatgaccaaaatcccttaacgtgagttttcgttccactgagcgtcagacccccatcagtgaccaaacaggaaaaaaccgcccttaacatggcccgctttatcagaagccagacattaacgcttctggagaaactcaacgagctggacgcggatgaacaggcagacatctgtgaatcgcttcacgaccacgctgatgagctttaccgcagctgcctcgcgcgtttcggtgatgacggtgaaaacctctgacacatgcagctcccggagacggtcacagcttgtctgtaagcggatgccgggagcagacaagcccgtcagggcgcgtcagcgggtgttggcgggtgtcggggcgcagccatgacccagtcacgtagcgatagcggagtgtatactggcttaactatgcggcatcagagcagattgtactgagagtgcaccatatgcggtgtgaaataccgcacagatgcgtaaggagaaaataccgcatcaggcgctcttccgcttcctcgctcactgactcgctgcgctcggtcgttcggctgcggcgagcggtatcagctcactcaaaggcggtaatacggttatccacagaatcaggggataacgcaggaaagaacatgtgagcaaaaggccagcaaaaggccaggaaccgtaaaaaggccgcgttgctggcgtttttccataggctccgcccccctgacgagcatcacaaaaatcgacgctcaagtcagaggtggcgaaacccgacaggactataaagataccaggcgtttccccctggaagctccctcgtgcgctctcctgttccgaccctgccgcttaccggatacctgtccgcctttctcccttcgggaagcgtggcgctttctcatagctcacgctgtaggtatctcagttcggtgtaggtcgttcgctccaagctgggctgtgtgcacgaaccccccgttcagcccgaccgctgcgccttatccggtaactatcgtcttgagtccaacccggtaagacacgacttatcgccactggcagcagccactggtaacaggattagcagagcgaggtatgtaggcggtgctacagagttcttgaagtggtggcctaactacggctacactagaaggacagtatttggtatctgcgctctgctgaagccagttaccttcggaaaaagagttggtagctcttgatccggcaaacaaaccaccgctggtagcggtggtttttttgtttgcaagcagcagattacgcgcagaaaaaaaggatctcaagaagatcctttgatc

SEQ ID NO: 3 - protein, 371 aa, human
MGSDVRDLNALLPAVPSLGGGGGCALPVSGAAQWAPVLDFAPPGASAYGSLGGPAPPPAPPPPPPPPPHSFIKQEPSWGGAEPHEEQCLSAFTVHFSGQFTGTAGACRYGPFGPPPPSQASSGQARMFPNAPYLPSCLESQPAIRNQGYSTVTFDGTPSYGHTPSHHAAQFPNHSFKHEDPMGQQGSLGEQQYSVPPPVYGCHTPTDSCTGSQALLLRTPYSSDNLYQMTSQLECMTWNQMNLGATLKGVAAGSSSSVKWTEGQSNHSTGYESDNHTTPILCGAQYRIHTHGVFRGIQDVRRVPGVAPTLVRSASETSEKRPFMCAYPGCNKRYFKLSHLQMHSRKHTGEKPYQCDFKDCERRFSRSDQLK

SEQ ID NO: 4 - protein, 630 aa, human
MALPTARPLLGSCGTPALGSLLFLLFSLGWVQPSRTLAGETGQEAAPLDGVLANPPNISSLSPRQLLGFPCAEVSGLSTERVRELAVALAQKNVKLSTEQLRCLAHRLSEPPEDLDALPLDLLLFLNPDAFSGPQACTRFFSRITKANVDLLPRGAPERQRLLPAALACWGVRGSLLSEADVRALGGLACDLPGRFVAESAEVLLPRLVSCPGPLDQDQQEAARAALQGGGPPYGPPSTWSVSTMDALRGLLPVLGQPIIRSIPQGIVAAWRQRSSRDPSWRQPERTILRPRFRREVEKTACPSGKKAREIDESLIFYKKWELEACVDAALLATQMDRVNAIPFTYEQLDVLKHKLDELYPQGYPESVIQHLGYLFLKMSPEDIRKWNVTSLETLKALLEVNKGHEMSPQAPRRPLPQVATLIDRFVKGRGQLDKDTLDTLTAFYPGYLCSLSPEELSSVPPSSIWAVRPQDLDTCDPRQLDVLYPKARLAFQNMNGSEYFVKIQSFLGGAPTEDLKALSQQNVSMDLATFMKLRTDAVLPLTVAEVQKLLGPHVEGLKAEERHRPVRDWILRQRQDDLDTLGLGLQGGIPNGYLVLDLSMQEALSGTPCLLGPGPVLTVLALLLASTLA

SEQ ID NO: 5 - protein, 702 aa, human
MESPSAPPHRWCIPWQRLLLTASLLTFWNPPTTAKLTIESTPFNVAEGKEVLLLVHNLPQHLFGYSWYKGERVDGNRQIIGYVIGTQQATPGPAYSGREIIYPNASLLIQNIIQNDTGFYTLHVIKSDLVNEEATGQFRVYPELPKPSISSNNSKPVEDKDAVAFTCEPETQDATYLWWVNNQSLPVSPRLQLSNGNRTLTLFNVTRNDTASYKCETQNPVSARRSDSVILNVLYGPDAPTISPLNTSYRSGENLNLSCHAASNPPAQYSWFVNGTFQQSTQELFIPNITVNNSGSYTCQAHNSDTGLNRTTVTTITVYAEPPKPFITSNNSNPVEDEDAVALTCEPEIQNTTYLWWVNNQSLPVSPRLQLSNDNRTLTLLSVTRNDVGPYECGIQNKLSVDHSDPVILNVLYGPDDPTISPSYTYYRPGVNLSLSCHAASNPPAQYSWLIDGNIQQHTQELFISNITEKNSGLYTCQANNSASGHSRTTVKTITVSAELPKPSISSNNSKPVEDKDAVAFTCEPEAQNTTYLWWVNGQSLPVSPRLQLSNGNRTLTLFNVTRNDARAYVCGIQNSVSANRSDPVTLDVLYGPDTPIISPPDSSYLSGANLNLSCHSASNPSPQYSWRINGIPQQHTQVLFIAKITPNNNGTYACFVSNLATGRNNSIVKSITVSASGTSPGLSAGATVGIMIGVLVGVALI

SEQ ID NO: 6 - protein, 561 aa, CMV
MESRGRRCPEMISVLGPISGHVLKAVFSRGDTPVLPHETRLLQTGIHVRVSQPSLILVSQYTPDSTPCHRGDNQLQVQHTYFTGSEVENVSVNVHNPTGRSICPSQEPMSIYVYALPLKMLNIPSINVHHYPSAAERKHRHLPVADAVIHASGKQMWQARLTVSGLAWTRQQNQWKEPDVYYTSAFVFPTKDVALRHVVCAHELVCSMENTRATKMQVIGDQYVKVYLESFCEDVPSGKLFMHVTLGSDVEEDLTMTRNPQPFMRPHERNGFTVLCPKNMIIKPGKISHIMLDVAFTSHEHFGLLCPKSIPGLSISGNLLMNGQQIFLEVQAIRETVELRQYDPVAALFFFDIDLLLQRGPQYSEHPTFTSQYRIQGKLEYRHTWDRHDEGAAQGDDDVWTSGSDSDEELVTTERKTPRVTGGGAMAGASTSAGRKRKSASSATACTAGVMTRGRLKAESTVAPEEDTDEDSDNEIHNPAVFTWPPWQAGILARNLVPMVATVQGQNLKYQEFFWDANDIYRIFAELEGVWQPAAQPKRRRHRQDALPGPCIASTPKKHRG

SEQ ID NO: 7 - protein, 561 aa, artificial
  mutated CMV pp65
MESRGRRCPEMISVLGPISGHVLKAVFSRGDTPVLPHETRLLQTGIHVRVSQPSLILVSQYTPDSTPCHRGDNQLQVQHTYFTGSEVENVSVNVHNPTGRSICPSQEPMSIYVYALPLKMLNIPSINVHHYPSAAERKHRHLPVADAVIHASGKQMWQARLTVSGLAWTRQQNQWKEPDVYYTSAFVFPTKDVALRHVVCAHELVCSMENTRATKMQVIGDQYVKVYLESFCEDVPSGKLFMHVTLGSDVEEDLTMTRNPQPFMRPHERNGFTVLCPKNMIIKPGKISHIMLDVAFTSHEHFGLLCPKSIPGLSISGNLLMNGQQIFLEVQAIRETVELRQYDPVAALFFFDIDLLLQRGPQYSEHPTFTSQYRIQGKLEYRHTWDRHDEGAAQGDDDVWTSGSDSDEELVTTERKTPRVTGGGAMAGASTSAGRNRKSASSATACTAGVMTRGRLKAESTVAPEEDTDEDSDNEIHNPAVFTWPPWQAGILARNLVPMVATVQGQNLKYQEFFWDANDIYRIFAELEGVWQPAAQPKRRRHRQDALPGPCIASTPKKHRG

SEQ ID NO: 8 - protein, 536 aa, artificial
  mutated CMV pp65
MESRGRRCPEMISVLGPISGHVLKAVFSRGDTPVLPHETRLLQTGIHVRVSQPSLILVSQYTPDSTPCHRGDNQLQVQHTYFTGSEVENVSVNVHNPTGRSICPSQEPMSIYVYALPLKMLNIPSINVHHYPSAAERKHRHLPVADAVIHASGKQMWQARLTVSGLAWTRQQNQWKEPDVYYTSAFVFPTKDVALRHVVCAHELVCSMENTRATKMQVIGDQYVKVYLESFCEDVPSGKLFMHVTLGSDVEEDLTMTRNPQPFMRPHERNGFTVLCPKNMIIKPGKISHIMLDVAFTSHEHFGLLCPKSIPGLSISGNLLMNGQQIFLEVQAIRETVELRQYDPVAALFFFDIDLLLQRGPQYSEHPTFTSQYRIQGKLEYRHTWDRHDEGAAQGDDDVWTSGSDSDEELVTTERKTPRVTGGGAMAGASTSAGRNRKSASSATACTAGVMTRGRLKAESTVAPEEDTDEDSDNEIHNPAVFTWPPWQAGILARNLVPMVATVQGQNLKYQEFFWDANDIYRIFAELEGVWQPAAQ

SEQ ID NO: 9 - DNA, 4071 bp, human
atgcagagcaaggtgctgctggccgtcgccctgtggctctgcgtggagacccgggccgcctctgtgggtttgcctagtgtttctcttgatctgcccaggctcagcatacaaaaagacatacttacaattaaggctaatacaactcttcaaattacttgcaggggacagagggacttggactggctttggcccaataatcagagtggcagtgagcaaagggtggaggtgactgagtgcagcgatggcctcttctgtaagacactcacaattccaaaagtgatcggaaatgacactggagcctacaagtgcttctaccgggaaactgacttggcctcggtcatttatgtctatgttcaagattacagatctccatttattgcttctgttagtgaccaacatggagtcgtgtacattactgagaacaaaaacaaaactgtggtgattccatgtctcgggtccatttcaaatctcaacgtgtcactttgtgcaagatacccagaaaagagatttgttcctgatggtaacagaatttcctgggacagcaagaagggctttactattcccagctacatgatcagctatgctggcatggtcttctgtgaagcaaaaattaatgatgaaagttaccagtctattatgtacatagttgtcgttgtagggtataggatttatgatgtggttctgagtccgtctcatggaattgaactatctgttggagaaaagcttgtcttaaattgtacagcaagaactgaactaaatgtggggattgacttcaactgggaatacccttcttcgaagcatcagcataagaaacttgtaaaccgagacctaaaaacccagtctgggagtgagatgaagaaatttttgagcaccttaactatagatggtgtaacccggagtgaccaaggattgtacacctgtgcagcatccagtgggctgatgaccaagaagaacagcacatttgtcagggtccatgaaaaaccttttgttgcttttggaagtggcatggaatctctggtggaagccacggtgggggagcgtgtcagaatccctgcgaagtaccttggttacccacccccagaaataaaatggtataaaaatggaataccccttgagtccaatcacacaattaaagcggggcatgtactgacgattatggaagtgagtgaaagagacacaggaaattacactgtcatccttaccaatcccatttcaaaggagaagcagagccatgtggtctctctggttgtgtatgtcccaccccagattggtgagaaatctctaatctctcctgtggattcctaccagtacggcaccactcaaacgctgacatgtacggtctatgccattcctcccccgcatcacatccactggtattggcagttggaggaagagtgcgccaacgagcccagccaagctgtctcagtgacaaacccatacccttgtgaagaatggagaagtgtggaggacttccagggaggaaataaaattgaagttaataaaaatcaatttgctctaattgaaggaaaaaacaaaactgtaagtacccttgttatccaagcggcaaatgtgtcagctttgtacaaatgtgaagcggtcaacaaagtcgggagaggagagagggtgatctccttccacgtgaccaggggtcctgaaattactttgcaacctgacatgcagcccactgagcaggagagcgtgtctttgtggtgcactgcagacagatctacgtttgagaacctcacatggtacaagcttggcccacagcctctgccaatccatgtgggagagttgcccacacctgtttgcaagaacttggatactctttggaaattgaatgccaccatgttctctaatagcacaaatgacattttgatcatggagcttaagaatgcatccttgcaggaccaaggagactatgtctgccttgctcaagacaggaagaccaagaaaagacattgcgtggtcaggcagctcacagtcctagagcgtgtggcacccacgatcacaggaaacctggagaatcagacgacaagtattggggaaagcatcgaagtctcatgcacggcatctgggaatccccctccacagatcatgtggtttaaagataatgagacccttgtagaagactcaggcattgtattgaaggatgggaaccggaacctcactatccgcagagtgaggaaggaggacgaaggcctctacacctgccaggcatgcagtgttcttggctgtgcaaaagtggaggcatttttcataatagaaggtgcccaggaaaagacgaacttggaaatcattattctagtaggcacggcggtgattgccatgttcttctggctacttcttgtcatcatcctacggaccgttaagcgggccaatggaggggaactgaagacaggctacttgtccatcgtcatggatccagatgaactcccattggatgaacattgtgaacgactgccttatgatgccagcaaatgggaattccccagagaccggctgaagctaggtaagcctcttggccgtggtgcctttggccaagtgattgaagcagatgcctttggaattgacaagacagcaacttgcaggacagtagcagtcaaaatgttgaaagaaggagcaacacacagtgagcatcgagctctcatgtctgaactcaagatcctcattcatattggtcaccatctcaatgtggtcaaccttctaggtgcctgtaccaagccaggagggccactcatggtgattgtggaattctgcaaatttggaaacctgtccacttacctgaggagcaagagaaatgaatttgtcccctacaagaccaaaggggcacgattccgtcaagggaaagactacgttggagcaatccctgtggatctgaaacggcgcttggacagcatcaccagtagccagagctcagccagctctggatttgtggaggagaagtccctcagtgatgtagaagaagaggaagctcctgaagatctgtataaggacttcctgaccttggagcatctcatctgttacagcttccaagtggctaagggcatggagttcttggcatcgcgaaagtgtatccacagggacctggcggcacgaaatatcctcttatcggagaagaacgtggttaaaatctgtgactttggcttggcccgggatatttataaagatccagattatgtcagaaaaggagatgctcgcctccctttgaaatggatggccccagaaacaatttttgacagagtgtacacaatccagagtgacgtctggtcttttggtgttttgctgtgggaaatattttccttaggtgcttctccatatcctggggtaaagattgatgaagaattttgtaggcgattgaaagaaggaactagaatgagggcccctgattatactacaccagaaatgtaccagaccatgctggactgctggcacggggagcccagtcagagacccacgttttcagagttggtggaacatttgggaaatctcttgcaagctaatgctcagcaggatggcaaagactacattgttcttccgatatcagagactttgagcatggaagaggattctggactctctctgcctacctcacctgtttcctgtatggaggaggaggaagtatgtgaccccaaattccattatgacaacacagcaggaatcagtcagtatctgcagaacagtaagcgaaagagccggcctgtgagtgtaaaaacatttgaagatatcccgttagaagaaccagaagtaaaagtaatcccagatgacaaccagacggacagtggtatggttcttgcctcagaagagctgaaaactttggaagacagaaccaaattatctccatcttttggtggaatggtgcccagcaaaagcagggagtctgtggcatctgaaggctcaaaccagacaagcggctaccagtccggatatcactccgatgacacagacaccaccgtgtactccagtgaggaagcagaacttttaaagctgatagagattggagtgcaaaccggtagcacagcccagattctccagcctgactcggggaccacactgagctctcctcctgtttaa

SEQ ID NO: 10 - DNA, 1116 bp, human
atggacttcctcttgctgcaggacccggcttccacgtgtgtcccggagccggcgtctcagcacacgctccgctccgggcctgggtgcctacagcagccagagcagcagggagtccgggacccgggcggcatctgggccaagttaggcgccgccgaggccagcgctgaacgtctccagggccggaggagccgcggggcgtccgggtctgagccgcagcaaatgggctccgacgtgcgggacctgaacgcgctgctgcccgccgtcccctccctgggtggcggcggcggctgtgccctgcctgtgagcggcgcggcgcagtgggcgccggtgctggactttgcgcccccgggcgcttcggcttacgggtcgttgggcggccccgcgccgccaccggctccgccgccacccccgccgccgccgcctcactccttcatcaaacaggagccgagctggggcggcgcggagccgcacgaggagcagtgcctgagcgccttcactgtccacttttccggccagttcactggcacagccggagcctgtcgctacgggcccttcggtcctcctccgcccagccaggcgtcatccggccaggccaggatgtttcctaacgcgccctacctgcccagctgcctggagagccagcccgctattcgcaatcagggttacagcacggtcaccttcgacgggacgcccagctacggtcacacgccctcgcaccatgcggcgcagttccccaaccactcattcaagcatgaggatcccatgggccagcagggctcgctgggtgagcagcagtactcggtgccgcccccggtctatggctgccacacccccaccgacagctgcaccggcagccaggctttgctgctgaggacgccctacagcagtgacaatttataccaaatgacatcccagcttgaatgcatgacctggaatcagatgaacttaggagccaccttaaagggagttgctgctgggagctccagctcagtgaaatggacagaagggcagagcaaccacagcacagggtacgagagcgataaccacacaacgcccatcctctgcggagcccaatacagaatacacacgcacggtgtcttcagaggcattcagtga

SEQ ID NO: 11 - DNA, 1893 bp, human
atggccttgccaacggctcgacccctgttggggtcctgtgggacccccgccctcggcagcctcctgttcctgctcttcagcctcggatgggtgcagccctccaggaccctggctggagagacagggcaggaggctgcgcccctggacggagtcctggccaacccacctaacatttccagcctctcccctcgccaactccttggcttcccgtgtgcggaggtgtccggcctgagcacggagcgtgtccgggagctggctgtggccttggcacagaagaatgtcaagctctcaacagagcagctgcgctgtctggctcaccggctctctgagccccccgaggacctggacgccctcccattggacctgctgctattcctcaacccagatgcgttctcggggccccaggcctgcacccgtttcttctcccgcatcacgaaggccaatgtggacctgctcccgaggggggctcccgagcgacagcggctgctgcctgcggctctggcctgctggggtgtgcgggggtctctgctgagcgaggctgatgtgcgggctctgggaggcctggcttgcgacctgcctgggcgctttgtggccgagtcggccgaagtgctgctaccccggctggtgagctgcccgggacccctggaccaggaccaacaggaggcagccagggcggctctgcagggcgggggacccccctacggccccccgtcgacatggtctgtctccacgatggacgctctgcggggcctgctgcccgtgctgggccagcccatcatccgcagcatcccgcagggcatcgtggccgcgtggcggcaacgctcctctcgggacccatcctggcggcagcctgaacggaccatcctccggccgcggttccggcgggaagtggagaagacagcctgtccttcaggcaagaaggcccgcgagatagacgagagcctcatcttctacaagaagtgggagctggaagcctgcgtggatgcggccctgctggccacccagatggaccgcgtgaacgccatccccttcacctacgagcagctggacgtcctaaagcataaactggatgagctctacccacaaggttaccccgagtctgtgatccagcacctgggctacctcttcctcaagatgagccctgaggacattcgcaagtggaatgtgacgtccctggagaccctgaaggctttgcttgaagtcaacaaagggcacgaaatgagtcctcaggctcctcggcggcccctcccacaggtggccaccctgatcgaccgctttgtgaagggaaggggccagctagacaaagacaccctagacaccctgaccgccttctaccctgggtacctgtgctccctcagccccgaggagctgagctccgtgccccccagcagcatctgggcggtcaggccccaggacctggacacgtgtgacccaaggcagctggacgtcctctatcccaaggcccgccttgctttccagaacatgaacgggtccgaatacttcgtgaagatccagtccttcctgggtggggcccccacggaggatttgaaggcgctcagtcagcagaatgtgagcatggacttggccacgttcatgaagctgcggacggatgcggtgctgccgttgactgtggctgaggtgcagaaacttctgggaccccacgtggagggcctgaaggcggaggagcggcaccgcccggtgcgggactggatcctacggcagcggcaggacgacctggacacgctggggctggggctacagggcggcatccccaacggctacctggtcctagacctcagcatgcaagaggccctctcggggacgccctgcctcctaggacctggacctgttctcaccgtcctggcactgctcctagcctccaccctggcctga

SEQ ID NO: 12 - DNA, 2109 bp, human
atggagtctccctcggcccctccccacagatggtgcatcccctggcagaggctcctgctcacagcctcacttctaaccttctggaacccgcccaccactgccaagctcactattgaatccacgccgttcaatgtcgcagaggggaaggaggtgcttctacttgtccacaatctgccccagcatctttttggctacagctggtacaaaggtgaaagagtggatggcaaccgtcaaattataggatatgtaataggaactcaacaagctaccccagggcccgcatacagtggtcgagagataatataccccaatgcatccctgctgatccagaacatcatccagaatgacacaggattctacaccctacacgtcataaagtcagatcttgtgaatgaagaagcaactggccagttccgggtatacccggagctgcccaagccctccatctccagcaacaactccaaacccgtggaggacaaggatgctgtggccttcacctgtgaacctgagactcaggacgcaacctacctgtggtgggtaaacaatcagagcctcccggtcagtcccaggctgcagctgtccaatggcaacaggaccctcactctattcaatgtcacaagaaatgacacagcaagctacaaatgtgaaacccagaacccagtgagtgccaggcgcagtgattcagtcatcctgaatgtcctctatggcccggatgcccccaccatttcccctctaaacacatcttacagatcaggggaaaatctgaacctctcctgccacgcagcctctaacccacctgcacagtactcttggtttgtcaatgggactttccagcaatccacccaagagctctttatccccaacatcactgtgaataatagtggatcctatacgtgccaagcccataactcagacactggcctcaataggaccacagtcacgacgatcacagtctatgcagagccacccaaacccttcatcaccagcaacaactccaaccccgtggaggatgaggatgctgtagccttaacctgtgaacctgagattcagaacacaacctacctgtggtgggtaaataatcagagcctcccggtcagtcccaggctgcagctgtccaatgacaacaggaccctcactctactcagtgtcacaaggaatgatgtaggaccctatgagtgtggaatccagaacaaattaagtgttgaccacagcgacccagtcatcctgaatgtcctctatggcccagacgaccccaccatttccccctcatacacctattaccgtccaggggtgaacctcagcctctcctgccatgcagcctctaacccacctgcacagtattcttggctgattgatgggaacatccagcaacacacacaagagctctttatctccaacatcactgagaagaacagcggactctatacctgccaggccaataactcagccagtggccacagcaggactacagtcaagacaatcacagtctctgcggagctgcccaagccctccatctccagcaacaactccaaacccgtggaggacaaggatgctgtggccttcacctgtgaacctgaggctcagaacacaacctacctgtggtgggtaaatggtcagagcctcccagtcagtcccaggctgcagctgtccaatggcaacaggaccctcactctattcaatgtcacaagaaatgacgcaagagcctatgtatgtggaatccagaactcagtgagtgcaaaccgcagtgacccagtcaccctggatgtcctctatgggccggacacccccatcatttcccccccagactcgtcttacctttcgggagcgaacctcaacctctcctgccactcggcctctaacccatccccgcagtattcttggcgtatcaatgggataccgcagcaacacacacaagttctctttatcgccaaaatcacgccaaataataacgggacctatgcctgttttgtctctaacttggctactggccgcaataattccatagtcaagagcatcacagtctctgcatctggaacttctcctggtctctcagctggggccactgtcggcatcatgattggagtgctggttggggttgctctgatatag

SEQ ID NO: 13 - DNA, 1683 bp, CMV
atggaatccagggggaggaggtgtccggagatgatctcagtcctcggaccgattagcggtcacgtgctcaaagcggtcttcagcagaggagacactccggtgctgccgcacgaaacaaggctccttcagacggggatacacgtgcgtgtgagtcagcccagcctgatcctcgtgtctcaatacacccctgacagcactccctgtcacagaggggacaaccaactccaggtccagcacacctacttcactgggagcgaggtcgagaacgtcagcgtgaacgtgcacaaccccacgggaagatcaatctgccctagccaggagcccatgagcatctacgtgtacgccctcccgctcaagatgctcaacatcccctccatcaacgtccaccactatccctccgctgccgaacgtaaacaccgacacttgccagttgcggacgccgtgatacacgcttcagggaagcagatgtggcaagccaggcttactgtgagtggactcgcctggactaggcaacagaaccagtggaaggagcccgacgtgtactacaccagcgccttcgtgttccccacaaaagacgtcgcgctgcgacatgtggtgtgcgctcacgaactggtgtgcagcatggagaacacgcgagcgaccaagatgcaggtgatcggtgaccagtacgtcaaggtgtacctggagagcttctgcgaggatgtcccgtccggaaagctgttcatgcacgtgaccctgggcagtgacgttgaggaagacctgaccatgacgcgtaacccgcagcctttcatgagaccgcacgagaggaacggattcaccgtcctgtgcccgaagaacatgatcatcaagcccggcaagatcagccacatcatgctcgacgtcgccttcacctctcacgaacacttcgggctgctgtgtccgaagagcattccgggtctgagcatctcaggcaacctgctgatgaacgggcagcagatcttcctggaagtgcaggccataagggagaccgtggaactgaggcagtacgatcctgtggctgccctgttcttcttcgacatcgacctcttgctgcaaaggggtccacagtatagcgaacaccccaccttcacctcccagtaccgtatccagggcaagctggagtaccgacacacttgggataggcacgacgagggtgccgctcaaggtgacgacgatgtttggactagcggctctgatagcgacgaagagctggtgaccactgagcgcaaaactccaagagttacgggcggcggcgcaatggctggcgcctctacttccgcgggaaggaaaaggaaaagcgcgtctagcgcaactgcatgcactgccggtgtgatgacaagggggagactgaaggccgagagtacagtggctccggaagaggataccgacgaggactctgacaacgagatccacaaccccgcagtgtttacgtggccaccttggcaagccggcatccttgctagaaacctggtgcccatggtggccacagtccaaggccagaacctgaagtaccaggagttcttctgggacgccaacgacatctaccgtatcttcgccgaacttgaaggcgtctggcagccggcggctcaacccaaaaggagacgtcacagacaggacgcgcttcccggaccctgtattgcctctacccccaagaaacaccggggc

SEQ ID NO: 14 - DNA, 1683 bp, artificial
  mutated CMV pp65 cDNA
atggaatccagggggaggaggtgtccggagatgatctcagtcctcggaccgattagcggtcacgtgctcaaagcggtcttcagcagaggagacactccggtgctgccgcacgaaacaaggctccttcagacggggatacacgtgcgtgtgagtcagcccagcctgatcctcgtgtctcaatacacccctgacagcactccctgtcacagaggggacaaccaactccaggtccagcacacctacttcactgggagcgaggtcgagaacgtcagcgtgaacgtgcacaaccccacgggaagatcaatctgccctagccaggagcccatgagcatctacgtgtacgccctcccgctcaagatgctcaacatcccctccatcaacgtccaccactatccctccgctgccgaacgtaaacaccgacacttgccagttgcggacgccgtgatacacgcttcagggaagcagatgtggcaagccaggcttactgtgagtggactcgcctggactaggcaacagaaccagtggaaggagcccgacgtgtactacaccagcgccttcgtgttccccacaaaagacgtcgcgctgcgacatgtggtgtgcgctcacgaactggtgtgcagcatggagaacacgcgagcgaccaagatgcaggtgatcggtgaccagtacgtcaaggtgtacctggagagcttctgcgaggatgtcccgtccggaaagctgttcatgcacgtgaccctgggcagtgacgttgaggaagacctgaccatgacgcgtaacccgcagcctttcatgagaccgcacgagaggaacggattcaccgtcctgtgcccgaagaacatgatcatcaagcccggcaagatcagccacatcatgctcgacgtcgccttcacctctcacgaacacttcgggctgctgtgtccgaagagcattccgggtctgagcatctcaggcaacctgctgatgaacgggcagcagatcttcctggaagtgcaggccataagggagaccgtggaactgaggcagtacgatcctgtggctgccctgttcttcttcgacatcgacctcttgctgcaaaggggtccacagtatagcgaacaccccaccttcacctcccagtaccgtatccagggcaagctggagtaccgacacacttgggataggcacgacgagggtgccgctcaaggtgacgacgatgtttggactagcggctctgatagcgacgaagagctggtgaccactgagcgcaaaactccaagagttacgggcggcggcgcaatggctggcgcctctacttccgcgggaaggaacaggaaaagcgcgtctagcgcaactgcatgcactgccggtgtgatgacaagggggagactgaaggccgagagtacagtggctccggaagaggataccgacgaggactctgacaacgagatccacaaccccgcagtgtttacgtggccaccttggcaagccggcatccttgctagaaacctggtgcccatggtggccacagtccaaggccagaacctgaagtaccaggagttcttctgggacgccaacgacatctaccgtatcttcgccgaacttgaaggcgtctggcagccggcggctcaacccaaaaggagacgtcacagacaggacgcgcttcccggaccctgtattgcctctacccccaagaaacaccggggc

SEQ ID NO: 15 - DNA, 1608 bp, artificial
  mutated CMV pp65 cDNA
atggaatccagggggaggaggtgtccggagatgatctcagtcctcggaccgattagcggtcacgtgctcaaagcggtcttcagcagaggagacactccggtgctgccgcacgaaacaaggctccttcagacggggatacacgtgcgtgtgagtcagcccagcctgatcctcgtgtctcaatacacccctgacagcactccctgtcacagaggggacaaccaactccaggtccagcacacctacttcactgggagcgaggtcgagaacgtcagcgtgaacgtgcacaaccccacgggaagatcaatctgccctagccaggagcccatgagcatctacgtgtacgccctcccgctcaagatgctcaacatcccctccatcaacgtccaccactatccctccgctgccgaacgtaaacaccgacacttgccagttgcggacgccgtgatacacgcttcagggaagcagatgtggcaagccaggcttactgtgagtggactcgcctggactaggcaacagaaccagtggaaggagcccgacgtgtactacaccagcgccttcgtgttccccacaaaagacgtcgcgctgcgacatgtggtgtgcgctcacgaactggtgtgcagcatggagaacacgcgagcgaccaagatgcaggtgatcggtgaccagtacgtcaaggtgtacctggagagcttctgcgaggatgtcccgtccggaaagctgttcatgcacgtgaccctgggcagtgacgttgaggaagacctgaccatgacgcgtaacccgcagcctttcatgagaccgcacgagaggaacggattcaccgtcctgtgcccgaagaacatgatcatcaagcccggcaagatcagccacatcatgctcgacgtcgccttcacctctcacgaacacttcgggctgctgtgtccgaagagcattccgggtctgagcatctcaggcaacctgctgatgaacgggcagcagatcttcctggaagtgcaggccataagggagaccgtggaactgaggcagtacgatcctgtggctgccctgttcttcttcgacatcgacctcttgctgcaaaggggtccacagtatagcgaacaccccaccttcacctcccagtaccgtatccagggcaagctggagtaccgacacacttgggataggcacgacgagggtgccgctcaaggtgacgacgatgtttggactagcggctctgatagcgacgaagagctggtgaccactgagcgcaaaactccaagagttacgggcggcggcgcaatggctggcgcctctacttccgcgggaaggaacaggaaaagcgcgtctagcgcaactgcatgcactgccggtgtgatgacaagggggagactgaaggccgagagtacagtggctccggaagaggataccgacgaggactctgacaacgagatccacaaccccgcagtgtttacgtggccaccttggcaagccggcatccttgctagaaacctggtgcccatggtggccacagtccaaggccagaacctgaagtaccaggagttcttctgggacgccaacgacatctaccgtatcttcgccgaacttgaaggcgtctggcagccggcggctcaa